European Patent Specification EP 3 600 257 B1, published May 10, 2023. Title: Alkaline Phosphatase Formulations. Applicant: Synthetic Biologics, Inc. Application PCT/US18/23327. The sequence listing filed with the application follows.

SEQUENCE LISTING (39 sequences)

SEQ ID NO: 1 - protein, 528 aa, Artificial Sequence
  Synthetic polypeptide
MQGPWVLLLLGLRLQLSLGVIPAEEENPAFWNRQAAEALDAAKKLQPIQKVAKNLILFLGDGLGVPTVTATRILKGQKNGKLGPETPLAMDRFPYLALSKTYNVDRQVPDSAATATAYLCGVKANFQTIGLSAAARFNQCNTTRGNEVISVMNRAKQAGKSVGVVTTTRVQHASPAGTYAHTVNRNWYSDADMPASARQEGCQDIATQLISNMDIDVILGGGRKYMFPMGTPDPEYPADASQNGIRLDGKNLVQEWLAKHQGAWYVWNRTELMQASLDQSVTHLMGLFEPGDTKYEIHRDPTLDPSLMEMTEAALRLLSRNPRGFYLFVEGGRIDHGHHEGVAYQALTEAVMFDDAIERAGQLTSEEDTLTLVTADHSHVFSFGGYTLRGSSIFGLAPSKAQDSKAYTSILYGNGPGYVFNSGVRPDVNESESGSPDYQQQAAVPLSSETHGGEDVAVFARGPQAHLVHGVQEQSFVAHVMAFAACLEPYTACDLAPPACTTDAAHPVAASLPLLAGTLLLLGASAAP

SEQ ID NO: 2 - protein, 533 aa, Artificial Sequence
  Synthetic polypeptide
MQGACVLLLLGLHLQLSLGLIPAEEENPAFWNRQAAQALDVAKKLQPIQTAAKNVILFLGDGMGVPTVTATRILKGQMNGKLGPETPLAMDQFPYVALSKTYNVDRQVPDSAGTATAYLCGVKGNYRTIGVSAAARYNQCNTTRGNEVTSVINRAKKAGKAVGVVTTTRVQHASPAGAYAHTVNRNWYSDADLPADAQKNGCQDIAAQLVYNMDIDVILGGGRMYMFPEGTPDPEYPDDASVNGVRKDKQNLVQEWQAKHQGAQYVWNRTALLQAADDSSVTHLMGLFEPADMKYNVQQDHTKDPTLAEMTEAALQVLSRNPRGFYLFVEGGRIDHGHHDGKAYMALTEAIMFDNAIAKANELTSELDTLILVTADHSHVFSFGGYTLRGTSIFGLAPGKALDSKSYTSILYGNGPGYALGGGSRPDVNGSTSEEPSYRQQAAVPLASETHGGEDVAVFARGPQAHLVHGVQEETFVAHIMAFAGCVEPYTDCNLPAPATATSIPDAAHLAASPPPLALLAGAMLLLLAPTLY

SEQ ID NO: 3 - protein, 530 aa, Artificial Sequence
  Synthetic polypeptide
MQWACVLLLLGLWLQLSLTFIPAEEEDPAFWNRQAAQALDVAKKLQPIQTAAKNVILFLGDGMGVPTVTATRILKGQMNGKLGPETPLAMDQFPYVALSKTYNVDRQVPDSAGTATAYLCGVKGNYKTIGVSAAARYNQCNTTSGNEVTSVMNRAKKAGKSVGVVTTSRVQHASPAGAYAHTVNRNWYSDADLPADAQTYGCQDIATQLVNNMDIDVILGGGRMYMFPEGTPDPEYPYDVNQTGVRKDKRNLVQEWQAKHQGAQYVWNRTELLQAANDPSVTHLMGLFEPADMKYNVQQDPTKDPTLEEMTEAALQVLSRNPQGFYLFVEGGRIDHGHHEGKAYMALTDTVMFDNAIAKANELTSELDTLILATADHSHVFSFGGYTLRGTSIFGLAPSKASDNKSYTSILYGNGPGYVLGGGLRPDVNDSISEDPSYRQQAAVPLSSESHGGEDVAVFARGPQAHLVHGVQEETFVAHVMAFAGCVEPYTDCNLPAPSGLSDAAHLAASPPSLALLAGAMLLLLAPALY

SEQ ID NO: 4 - protein, 503 aa, Artificial Sequence
  Synthetic polypeptide
MQGPWVLLLLGLRLQLSLGVIPAEEENPAFWNRQAAEALDAAKKLQPIQKVAKNLILFLGDGLGVPTVTATRILKGQKNGKLGPETPLAMDRFPYLALSKTYNVDRQVPDSAATATAYLCGVKANFQTIGLSAAARFNQCNTTRGNEVISVMNRAKQAGKSVGVVTTTRVQHASPAGTYAHTVNRNWYSDADMPASARQEGCQDIATQLISNMDIDVILGGGRKYMFPMGTPDPEYPADASQNGIRLDGKNLVQEWLAKHQGAWYVWNRTELMQASLDQSVTHLMGLFEPGDTKYEIHRDPTLDPSLMEMTEAALRLLSRNPRGFYLFVEGGRIDHGHHEGVAYQALTEAVMFDDAIERAGQLTSEEDTLTLVTADHSHVFSFGGYTLRGSSIFGLAPSKAQDSKAYTSILYGNGPGYVFNSGVRPDVNESESGSPDYQQQAAVPLSSETHGGEDVAVFARGPQAHLVHGVQEQSFVAHVMAFAACLEPYTACDLAPPAGTTD

SEQ ID NO: 5 - protein, 506 aa, Artificial Sequence
  Synthetic polypeptide
MQGACVLLLLGLHLQLSLGLIPAEEENPAFWNRQAAQALDVAKKLQPIQTAAKNVILFLGDGMGVPTVTATRILKGQMNGKLGPETPLAMDQFPYVALSKTYNVDRQVPDSAGTATAYLCGVKGNYRTIGVSAAARYNQCNTTRGNEVTSVINRAKKAGKAVGVVTTTRVQHASPAGAYAHTVNRNWYSDADLPADAQKNGCQDIAAQLVYNMDIDVILGGGRMYMFPEGTPDPEYPDDASVNGVRKDKQNLVQEWQAKHQGAQYVWNRTALLQAADDSSVTHLMGLFEPADMKYNVQQDHTKDPTLAEMTEAALQVLSRNPRGFYLFVEGGRIDHGHHDGKAYMALTEAIMFDNAIAKANELTSELDTLILVTADHSHVFSFGGYTLRGTSIFGLAPGKALDSKSYTSILYGNGPGYALGGGSRPDVNGSTSEEPSYRQQAAVPLASETHGGEDVAVFARGPQAHLVHGVQEETFVAHIMAFAGCVEPYTDCNLPAPATATSIPD

SEQ ID NO: 6 - protein, 503 aa, Artificial Sequence
  Synthetic polypeptide
MQWACVLLLLGLWLQLSLTFIPAEEEDPAFWNRQAAQALDVAKKLQPIQTAAKNVILFLGDGMGVPTVTATRILKGQMNGKLGPETPLAMDQFPYVALSKTYNVDRQVPDSAGTATAYLCGVKGNYKTIGVSAAARYNQCNTTSGNEVTSVMNRAKKAGKSVGVVTTSRVQHASPAGAYAHTVNRNWYSDADLPADAQTYGCQDIATQLVNNMDIDVILGGGRMYMFPEGTPDPEYPYDVNQTGVRKDKRNLVQEWQAKHQGAQYVWNRTELLQAANDPSVTHLMGLFEPADMKYNVQQDPTKDPTLEEMTEAALQVLSRNPQGFYLFVEGGRIDHGHHEGKAYMALTDTVMFDNAIAKANELTSELDTLILATADHSHVFSFGGYTLRGTSIFGLAPSKASDNKSYTSILYGNGPGYVLGGGLRPDVNDSISEDPSYRQQAAVPLSSESHGGEDVAVFARGPQAHLVHGVQEETFVAHVMAFAGCVEPYTDCNLPAPSGLSD

SEQ ID NO: 7 - protein, 508 aa, Artificial Sequence
  Synthetic polypeptide
MQWACVLLLLGLWLQLSLTFIPAEEEDPAFWNRQAAQALDVAKKLQPIQTAAKNVILFLGDGMGVPTVTATRILKGQMNGKLGPETPLAMDQFPYVALSKTYNVDRQVPDSAGTATAYLCGVKGNYKTIGVSAAARYNQCNTTSGNEVTSVMNRAKKAGKSVGVVTTSRVQHASPAGAYAHTVNRNWYSDADLPADAQTYGCQDIATQLVNNMDIDVILGGGRMYMFPEGTPDPEYPYDVNQTGVRKDKRNLVQEWQAKHQGAQYVWNRTELLQAANDPSVTHLMGLFEPADMKYNVQQDPTKDPTLEEMTEAALQVLSRNPQGFYLFVEGGRIDHGHHEGKAYMALTDTVMFDNAIAKANELTSELDTLILATADHSHVFSFGGYTLRGTSIFGLAPSKASDNKSYTSILYGNGPGYVLGGGLRPDVNDSISEDPSYRQQAAVPLSSESHGGEDVAVFARGPQAHLVHGVQEETFVAHVMAFAGCVEPYTDCNLPAPSGLSDAAHLA

SEQ ID NO: 8 - protein, 754 aa, Artificial Sequence
  Synthetic polypeptide
MQGACVLLLLGLHLQLSLGLIPAEEENPAFWNRQAAQALDVAKKLQPIQTAAKNVILFLGDGMGVPTVTATRILKGQMNGKLGPETPLAMDQFPYVALSKTYNVDRQVPDSAGTATAYLCGVKGNYRTIGVSAAARYNQCNTTRGNEVTSVINRAKKAGKAVGVVTTTRVQHASPAGAYAHTVNRNWYSDADLPADAQKNGCQDIAAQLVYNMDIDVILGGGRMYMFPEGTPDPEYPDDASVNGVRKDKQNLVQEWQAKHQGAQYVWNRTALLQAADDSSVTHLMGLFEPADMKYNVQQDHTKDPTLAEMTEAALQVLSRNPRGFYLFVEGGRIDHGHHDGKAYMALTEAIMFDNAIAKANELTSELDTLILVTADHSHVFSFGGYTLRGTSIFGLAPGKALDSKSYTSILYGNGPGYALGGGSRPDVNGSTSEEPSYRQQAAVPLASETHGGEDVAVFARGPQAHLVHGVQEETFVAHIMAFAGCVEPYTDCNLPAPATATSIPDGGSGGSGGGGSGGGGSEPKSCDKTHTCPPCPAPELLGGPSVFLFPPKPKDTLMISRTPEVTCVVVDVSHEDPQVKFNWYVDGVQVHNAKTKPREQQYNSTYRVVSVLTVLHQNWLDGKEYKCKVSNKALPAPIEKTISKAKGQPREPQVYTLPPSREEMTKNQVSLTCLVKGFYPSDIAVEWESNGQPENNYKTTPPVLDSDGSFFLYSKLTVDKSRWQQGNVFSCSVMHEALHNHYTQKSLSLSPGK

SEQ ID NO: 9 - protein, 751 aa, Artificial Sequence
  Synthetic polypeptide
MQWACVLLLLGLWLQLSLTFIPAEEEDPAFWNRQAAQALDVAKKLQPIQTAAKNVILFLGDGMGVPTVTATRILKGQMNGKLGPETPLAMDQFPYVALSKTYNVDRQVPDSAGTATAYLCGVKGNYKTIGVSAAARYNQCNTTSGNEVTSVMNRAKKAGKSVGVVTTSRVQHASPAGAYAHTVNRNWYSDADLPADAQTYGCQDIATQLVNNMDIDVILGGGRMYMFPEGTPDPEYPYDVNQTGVRKDKRNLVQEWQAKHQGAQYVWNRTELLQAANDPSVTHLMGLFEPADMKYNVQQDPTKDPTLEEMTEAALQVLSRNPQGFYLFVEGGRIDHGHHEGKAYMALTDTVMFDNAIAKANELTSELDTLILATADHSHVFSFGGYTLRGTSIFGLAPSKASDNKSYTSILYGNGPGYVLGGGLRPDVNDSISEDPSYRQQAAVPLSSESHGGEDVAVFARGPQAHLVHGVQEETFVAHVMAFAGCVEPYTDCNLPAPSGLSDGGSGGSGGGGSGGGGSEPKSCDKTHTCPPCPAPELLGGPSVFLFPPKPKDTLMISRTPEVTCVVVDVSHEDPQVKFNWYVDGVQVHNAKTKPREQQYNSTYRVVSVLTVLHQNWLDGKEYKCKVSNKALPAPIEKTISKAKGQPREPQVYTLPPSREEMTKNQVSLTCLVKGFYPSDIAVEWESNGQPENNYKTTPPVLDSDGSFFLYSKLTVDKSRWQQGNVFSCSVMHEALHNHYTQKSLSLSPGK

SEQ ID NO: 10 - protein, 539 aa, Artificial Sequence
  Synthetic polypeptide
MQWACVLLLLGLWLQLSLTFIPAEEEDPAFWNRQAAQALDVAKKLQPIQTAAKNVILFLGDGMGVPTVTATRILKGQMNGKLGPETPLAMDQFPYVALSKTYNVDRQVPDSAGTATAYLCGVKGNYKTIGVSAAARYNQCNTTSGNEVTSVMNRAKKAGKSVGVVTTSRVQHASPAGAYAHTVNRNWYSDADLPADAQTYGCQDIATQLVNNMDIDVILGGGRMYMFPEGTPDPEYPYDVNQTGVRKDKRNLVQEWQAKHQGAQYVWNRTELLQAANDPSVTHLMGLFEPADMKYNVQQDPTKDPTLEEMTEAALQVLSRNPQGFYLFVEGGRIDHGHHEGKAYMALTDTVMFDNAIAKANELTSELDTLILATADHSHVFSFGGYTLRGTSIFGLAPSKASDNKSYTSILYGNGPGYVLGGGLRPDVNDSISEDPSYRQQAAVPLSSESHGGEDVAVFARGPQAHLVHGVQEETFVAHVMAFAGCVEPYTDCNLEVLFQGPAPPAGTTDAAHPGRSVVPALLPLRAGTLLLLETATAP

SEQ ID NO: 11 - protein, 534 aa, Artificial Sequence
  Synthetic polypeptide
MQWACVLLLLGLWLQLSLTFIPAEEEDPAFWNRQAAQALDVAKKLQPIQTAAKNVILFLGDGMGVPTVTATRILKGQMNGKLGPETPLAMDQFPYVALSKTYNVDRQVPDSAGTATAYLCGVKGNYKTIGVSAAARYNQCNTTSGNEVTSVMNRAKKAGKSVGVVTTSRVQHASPAGAYAHTVNRNWYSDADLPADAQTYGCQDIATQLVNNMDIDVILGGGRMYMFPEGTPDPEYPYDVNQTGVRKDKRNLVQEWQAKHQGAQYVWNRTELLQAANDPSVTHLMGLFEPADMKYNVQQDPTKDPTLEEMTEAALQVLSRNPQGFYLFVEGGRIDHGHHEGKAYMALTDTVMFDNAIAKANELTSELDTLILATADHSHVFSFGGYTLRGTSIFGLAPSKASDNKSYTSILYGNGPGYVLGGGLRPDVNDSISEDPSYRQQAAVPLSSESHGGEDVAVFARGPQAHLVHGVQEETFVAHVMAFAGCVEPYTDCNLAPPAGTTDAAHPIEGRSVVPALLPLRAGTLLLLETATAP

SEQ ID NO: 12 - DNA, 1669 bp, Artificial Sequence
  Synthetic polynucleotide
atgcaggggccctgggtgctgctgctgctgggcctgaggctacagctctccctgggcgtcatcccaggtaatgaggctccccaagctgttccacacacagggcaccccctcagccaggctgacctgatctctactctccccctggccagctgaggaggagaacccggccttctggaaccgccaggcagctgaggccctggatgctgccaagaagctgcagcccatccagaaggtcgccaagaacctcatcctcttcctgggcgatgggttgggggtgcccacggtgacagccaccaggatcctaaaggggcagaagaatggcaaactggggcctgagacgcccctggccatggaccgcttcccatacctggctctgtccaagacatacaatgtggacagacaggtgccagacagcgcagccacagccacggcctacctgtgcggggtcaaggccaacttccagaccatcggcttgagtgcagccgcccgctttaaccagtgcaacacgacacgcggcaatgaggtcatctccgtgatgaaccgggccaagcaagcaggaaagtcagtaggagtggtgaccaccacacgggtgcagcacgcctcgccagccggcacctacgcacacacagtgaaccgcaactggtactcagatgctgacatgcctgcctcagcccgccaggaggggtgccaggacatcgccactcagctcatctccaacatggacattgacgtgatccttggcggaggccgcaagtacatgtttcccatggggaccccagaccctgagtacccagctgatgccagccagaatggaatcaggctggacgggaagaacctggtgcaggaatggctggcaaagcaccagggtgcctggtatgtgtggaaccgcactgagctcatgcaggcgtccctggaccagtctgtgacccatctcatgggcctctttgagcccggagacacgaaatatgagatccaccgagaccccacactggacccctccctgatggagatgacagaggctgccctgcgcctgctgagcaggaacccccgcggcttctacctctttgtggagggcggccgcatcgaccatggtcatcatgagggtgtggcttaccaggcactcactgaggcggtcatgttcgacgacgccattgagagggcgggccagctcaccagcgaggaggacacgctgaccctcgtcaccgctgaccactcccatgtcttctcctttggtggctacaccttgcgagggagctccatcttcgggttggcccccagcaaggctcaggacagcaaagcctacacgtccatcctgtacggcaatggcccgggctacgtgttcaactcaggcgtgcgaccagacgtgaatgagagcgagagcgggagccccgattaccagcagcaggcggcggtgcccctgtcgtccgagacccacggaggcgaagacgtggcggtgtttgcgcgcggcccgcaggcgcacctggtgcatggtgtgcaggagcagagcttcgtagcgcatgtcatggccttcgctgcctgtctggagccctacacggcctgcgacctggcgcctcccgcctgcaccaccgacgccgcgcacccagttgccgcgtcgctgccactgctggccgggaccctgctgctgctgggggcgtccgctgctccctga

SEQ ID NO: 13 - DNA, 1671 bp, Artificial Sequence
  Synthetic polynucleotide
atgcaggggccctgggtgctgctgctgctgggcctgaggctacagctctccctgggcgtcatcccagctgaggaggagaacccggccttctggaaccgccaggcagctgaggccctggatgctgccaagaagctgcagcccatccagaaggtcgccaagaacctcatcctcttcctgggcgatgggttgggggtgcccacggtgacagccaccaggatcctaaaggggcagaagaatggcaaactggggcctgagacgcccctggccatggaccgcttcccatacctggctctgtccaagacatacaatgtggacagacaggtgccagacagcgcagccacagccacggcctacctgtgcggggtcaaggccaacttccagaccatcggcttgagtgcagccgcccgctttaaccagtgcaacacgacacgcggcaatgaggtcatctccgtgatgaaccgggccaagcaagcaggaaagtcagtaggagtggtgaccaccacacgggtgcagcacgcctcgccagccggcacctacgcacacacagtgaaccgcaactggtactcagatgctgacatgcctgcctcagcccgccaggaggggtgccaggacatcgccactcagctcatctccaacatggacattgacgtgatccttggcggaggccgcaagtacatgtttcccatggggaccccagaccctgagtacccagctgatgccagccagaatggaatcaggctggacgggaagaacctggtgcaggaatggctggcaaagcaccagggtgcctggtatgtgtggaaccgcactgagctcatgcaggcgtccctggaccagtctgtgacccatctcatgggcctctttgagcccggagacacgaaatatgagatccaccgagaccccacactggacccctccctgatggagatgacagaggctgccctgcgcctgctgagcaggaacccccgcggcttctacctctttgtggagggcggccgcatcgaccatggtcatcatgagggtgtggcttaccaggcactcactgaggcggtcatgttcgacgacgccattgagagggcgggccagctcaccagcgaggaggacacgctgaccctcgtcaccgctgaccactcccatgtcttctcctttggtggctacaccttgcgagggagctccatcttcgggttggcccccagcaaggctcaggacagcaaagcctacacgtccatcctgtacggcaatggcccgggctacgtgttcaactcaggcgtgcgaccagacgtgaatgagagcgagagcgggagccccgattaccagcagcaggcggcggtgcccctgtcgtccgagacccacggaggcgaagacgtggcggtgtttgcgcgcggcccgcaggcgcacctggtgcatggtgtgcaggagcagagcttcgtagcgcatgtcatggccttcgctgcctgtctggagccctacacggcctgcgacctggcgcctcccgcctgcaccaccgacgccgcgcacccagttgccgcgtcgctgccactgctggccgggaccctgctgctgctgggggcgtccgctgctccctgatttactaaaaccttgaaataaaattgtaaaacatcagtttgaaggcctgactctcagggtagttcttttttaattctgggtttt

SEQ ID NO: 14 - DNA, 1672 bp, Artificial Sequence
  Synthetic polynucleotide
atgcagtgggcctgtgtgctgctgctgctgggcctgtggctacagctctccctcaccttcatcccaggtaatcaggcggctcccagcagcccctactcacaggggcggctctaggctgacctgaccaacactctccccttgggcagctgaggaggaagaccccgccttctggaaccgccaggcagcccaggcccttgatgtagccaagaagttgcagccgatccagacagctgccaagaatgtcatcctcttcttgggggatgggatgggggtgcctacggtgacagccactcggatcctaaaggggcagatgaatggtaagctgggacctgagacacccctggccatggaccagttcccatacgtggctctgtccaagacatacaacgtggacagacaggtgccagacagcgcaggcactgccactgcctacctgtgtggggtcaagggcaactacaaaaccattggtgtaagtgcagccgcccgctacaaccagtgcaacacaacaagtggcaatgaggtcacgtctgtgatgaaccgggccaagaaagcaggaaagtcagtgggagtggtgaccacctccagggtgcagcatgcctccccagccggtgcttatgcacacacggtgaaccgaaactggtactcagatgccgacctgcctgccgatgcacagacgtatggctgccaggacatcgccacacaactggtcaacaacatggatattgacgtgatcctgggtggaggccgaatgtacatgtttcctgaggggaccccggatcctgaatacccatacgatgtcaatcagactggagtccggaaggacaagcggaatctggtgcaggagtggcaggccaagcaccagggagcccagtatgtgtggaaccgcacggagctccttcaggcagccaatgaccccagtgtaacacacctcatgggcctctttgagccggcagacatgaagtataatgttcagcaagaccccaccaaggacccgaccctggaggagatgacggaggcggccctgcaagtgctgagcaggaacccccagggcttctacctcttcgtggagggaggccgcattgaccacggtcaccatgaaggcaaagcttatatggcactgactgatacagtcatgtttgacaatgccatcgccaaggctaacgagctcactagcgaactggacacgctgatccttgccactgcagaccactcccatgtcttctcttttggtggctacacactgcgtgggacctccattttcggtctggcccccagcaaggcctcagacaacaagtcctacacctccatcctctatggcaatggccctggctacgtgcttggtgggggcttaaggcccgatgttaatgacagcataagcgaggacccctcgtaccggcagcaggcggccgtgcccctgtctagtgagtcccacgggggcgaggacgtggcggtgttcgcgcgaggcccgcaggcgcacctggtgcacggcgtgcaggaggagaccttcgtggcgcacgtcatggcctttgcgggctgcgtggagccctacaccgactgcaatctgccggccccctctggcctctccgacgccgcgcacctggcggccagcccgccttcgctggcgctgctggccggggcgatgctgctgctgctggcgcctgccttgtactga

SEQ ID NO: 15 - DNA, 1869 bp, Artificial Sequence
  Synthetic polynucleotide
atgcagtgggcctgtgtgctgctgctgctgggcctgtggctacagctctccctcaccttcatcccagctgaggaggaagaccccgccttctggaaccgccaggcagcccaggcccttgatgtagccaagaagttgcagccgatccagacagctgccaagaatgtcatcctcttcttgggggatgggatgggggtgcctacggtgacagccactcggatcctaaaggggcagatgaatggtaagctgggacctgagacacccctggccatggaccagttcccatacgtggctctgtccaagacatacaacgtggacagacaggtgccagacagcgcaggcactgccactgcctacctgtgtggggtcaagggcaactacaaaaccattggtgtaagtgcagccgcccgctacaaccagtgcaacacaacaagtggcaatgaggtcacgtctgtgatgaaccgggccaagaaagcaggaaagtcagtgggagtggtgaccacctccagggtgcagcatgcctccccagccggtgcttatgcacacacggtgaaccgaaactggtactcagatgccgacctgcctgccgatgcacagacgtatggctgccaggacatcgccacacaactggtcaacaacatggatattgacgtgatcctgggtggaggccgaatgtacatgtttcctgaggggaccccggatcctgaatacccatacgatgtcaatcagactggagtccggaaggacaagcggaatctggtgcaggagtggcaggccaagcaccagggagcccagtatgtgtggaaccgcacggagctccttcaggcagccaatgaccccagtgtaacacacctcatgggcctctttgagccggcagacatgaagtataatgttcagcaagaccccaccaaggacccgaccctggaggagatgacggaggcggccctgcaagtgctgagcaggaacccccagggcttctacctcttcgtggagggaggccgcattgaccacggtcaccatgaaggcaaagcttatatggcactgactgatacagtcatgtttgacaatgccatcgccaaggctaacgagctcactagcgaactggacacgctgatccttgccactgcagaccactcccatgtcttctcttttggtggctacacactgcgtgggacctccattttcggtctggcccccagcaaggcctcagacaacaagtcctacacctccatcctctatggcaatggccctggctacgtgcttggtgggggcttaaggcccgatgttaatgacagcataagcgaggacccctcgtaccggcagcaggcggccgtgcccctgtctagtgagtcccacgggggcgaggacgtggcggtgttcgcgcgaggcccgcaggcgcacctggtgcacggcgtgcaggaggagaccttcgtggcgcacgtcatggcctttgcgggctgcgtggagccctacaccgactgcaatctgccggccccctctggcctctccgacgccgcgcacctggcggccagcccgccttcgctggcgctgctggccggggcgatgctgctgctgctggcgcctgccttgtactgaggggacccgggggtggggacacaggccccgccctccctgggaggcaggaagcagctctcaaataaactgttctaagtatgatacaggagtgatacatgtgtgaagagaagcccttaggtgggggcacagagtgtctgggtgaggggggtcagggtcacatcaggaggttagggaggggttgatgaagggctgacgttgagcaaagaccaaaggcaactcagaaggacagtggtgcaggactgggtgtggtcagcagggggactggttgggggatcc

SEQ ID NO: 16 - DNA, 1260 bp, Artificial Sequence
  Synthetic polynucleotide
aaaaaacaagacaaagctgagatcagaaatgtcattgtgatgataggcgacggcatggggacgccttacataagagcctaccgttccatgaaaaataacggtgacacaccgaataacccgaagttaacagaatttgaccggaacctgacaggcatgatgatgacgcatccggatgaccctgactataatattacagattcagcagcagccggaacagcattagcgacaggcgttaagacatataacaatgcaattggcgtcgataaaaacggaaaaaaagtgaaatctgtacttgaagaggccaaacagcaaggcaagtcaacagggcttgtcgccacgtctgaaattaaccacgccactccagccgcatatggcgcccacaatgaatcacggaaaaacatggaccaaatcgccaacagctatatggatgacaagataaaaggcaaacataaaatagacgtgctgctcggcggcggaaaatcttattttaaccgcaagaacagaaacttgacaaaggaattcaaacaagccggctacagctatgtgacaactaaacaagcattgaaaaaaaataaagatcagcaggtgctcgggcttttcgcagatggagggcttgctaaagcgctcgaccgtgacagtaaaacaccgtctctcaaagacatgacggtttcagcaattgatcgcctgaaccaaaataaaaaaggatttttcttgatggtcgaagggagccagattgactgggcggcccatgacaatgatacagtaggagccatgagcgaggttaaagattttgaacaggcctataaagccgcgattgaatttgcgaaaaaagacaaacatacacttgtgattgcaactgctgaccatacaaccggcggctttaccattggcgcaaacggggaaaagaattggcacgcagaaccgattctctccgctaagaaaacacctgaattcatggccaaaaaaatcagtgaaggcaagccggttaaagatgtgctcgcccgctatgccaatctgaaagtcacatctgaagaaatcaaaagcgttgaagcagctgcacaggctgacaaaagcaaaggggcctccaaagccatcatcaagatttttaatacccgctccaacagcggatggacgagtaccgatcataccggcgaagaagtaccggtatacgcgtacggccccggaaaagaaaaattccgcggattgattaacaatacggaccaggcaaacatcatatttaagattttaaaaactggaaaa

SEQ ID NO: 17 - protein, 420 aa, Artificial Sequence
  Synthetic polypeptide
KKQDKAEIRNVIVMIGDGMGTPYIRAYRSMKNNGDTPNNPKLTEFDRNLTGMMMTHPDDPDYNITDSAAAGTALATGVKTYNNAIGVDKNGKKVKSVLEEAKQQGKSTGLVATSEINHATPAAYGAHNESRKNMDQIANSYMDDKIKGKHKIDVLLGGGKSYFNRKNRNLTKEFKQAGYSYVTTKQALKKNKDQQVLGLFADGGLAKALDRDSKTPSLKDMTVSAIDRLNQNKKGFFLMVEGSQIDWAAHDNDTVGAMSEVKDFEQAYKAAIEFAKKDKHTLVIATADHTTGGFTIGANGEKNWHAEPILSAKKTPEFMAKKISEGKPVKDVLARYANLKVTSEEIKSVEAAAQADKSKGASKAIIKIFNTRSNSGWTSTDHTGEEVPVYAYGPGKEKFRGLINNTDQANIIFKILKTGK

SEQ ID NO: 18 - protein, 16 aa, Artificial Sequence
  Synthetic polypeptide
GGSGGSGGGGSGGGGS

SEQ ID NO: 19 - protein, 5 aa, Artificial Sequence
  Synthetic peptide
GGGGS

SEQ ID NO: 20 - protein, 10 aa, Artificial Sequence
  Synthetic peptide
GGGGSGGGGS

SEQ ID NO: 21 - protein, 15 aa, Artificial Sequence
  Synthetic peptide
GGGGSGGGGSGGGGS

SEQ ID NO: 22 - protein, 20 aa, Artificial Sequence
  Synthetic peptide
GGGGSGGGGSGGGGSGGGGS

SEQ ID NO: 23 - protein, 8 aa, Artificial Sequence
  Synthetic peptide
GGGGGGGG

SEQ ID NO: 24 - protein, 6 aa, Artificial Sequence
  Synthetic peptide
GGGGGG

SEQ ID NO: 25 - protein, 5 aa, Artificial Sequence
  Synthetic peptide
EAAAK

SEQ ID NO: 26 - protein, 10 aa, Artificial Sequence
  Synthetic peptide
EAAAKEAAAK

SEQ ID NO: 27 - protein, 15 aa, Artificial Sequence
  Synthetic peptide
EAAAKEAAAKEAAAK

SEQ ID NO: 28 - protein, 12 aa, Artificial Sequence
  Synthetic peptide
AEAAAKEAAAKA

SEQ ID NO: 29 - protein, 17 aa, Artificial Sequence
  Synthetic peptide
AEAAAKEAAAKEAAAKA

SEQ ID NO: 30 - protein, 22 aa, Artificial Sequence
  Synthetic peptide
AEAAAKEAAAKEAAAKEAAAKA

SEQ ID NO: 31 - protein, 27 aa, Artificial Sequence
  Synthetic peptide
AEAAAKEAAAKEAAAKEAAAKEAAAKA

SEQ ID NO: 32 - protein, 46 aa, Artificial Sequence
  Synthetic polypeptide
AEAAAKEAAAKEAAAKEAAAKALEAEAAAKEAAAKEAAAKEAAAKA

SEQ ID NO: 33 - protein, 5 aa, Artificial Sequence
  Synthetic peptide
PAPAP

SEQ ID NO: 34 - protein, 18 aa, Artificial Sequence
  Synthetic peptide
KESGSVSSEQLAQFRSLD

SEQ ID NO: 35 - protein, 14 aa, Artificial Sequence
  Synthetic peptide
EGKSSGSGSESKST

SEQ ID NO: 36 - protein, 12 aa, Artificial Sequence
  Synthetic peptide
GSAGSAAGSGEF

SEQ ID NO: 37 - DNA, 13 bp, Artificial Sequence
  Synthetic polynucleotide
gccgccaccatgg

SEQ ID NO: 38 - protein, 10 aa, Artificial Sequence
  Synthetic polymer.
ALLPLLAGTL

SEQ ID NO: 39 - protein, 10 aa, Artificial Sequence
  Synthetic polymer.
ALLPLRAGTL